European Patent Application EP 4 163 280 A1, published April 12, 2023. Title: PRODUCTION METHOD OF HETEROCYCLIC COMPOUND. Applicant: TAKEDA PHARMACEUTICAL COMPANY LIMITED. The sequence listing filed with the application follows.

SEQUENCE LISTING (1 sequence)

SEQ ID NO: 1 - DNA, 18 bp, Artificial Sequence
  linker sequence
ggaagtggctcaggtagc